European Patent Specification EP 3 610 030 B1, published August 7, 2024. Title: Methods for Variant Detection. Applicant: Integrated DNA Technologies, Inc. The sequence listing filed with the application follows.

SEQUENCE LISTING (218 sequences)

SEQ ID NO: 1 - DNA, 24 bp, Artificial Sequence
  Synthetic
gctgtgattttggtctagctacag

SEQ ID NO: 2 - DNA, 25 bp, Artificial Sequence
  Synthetic
gctgtgattttggtctagctacagt

SEQ ID NO: 3 - DNA, 25 bp, Artificial Sequence
  Synthetic
gctgtgattttggtctagctacaga

SEQ ID NO: 4 - DNA, 27 bp, Artificial Sequence
  Synthetic
  misc_feature (1)..(1): 5' 6-carboxyfluorescein
  misc_feature (9)..(10): internal ZEN quencher
  misc_feature (27)..(27): 3' Iowa Black fluorescence quencher
tcccatcagtttgaacagttgtctgga

SEQ ID NO: 5 - DNA, 31 bp, Artificial Sequence
  Synthetic
  misc_feature (26)..(26): RNA
  misc_feature (31)..(31): 3' C3 propanediol spacer block
gctgtgattttggtctagctacagtgaaatg

SEQ ID NO: 6 - DNA, 31 bp, Artificial Sequence
  Synthetic
  misc_feature (26)..(26): RNA
  misc_feature (31)..(31): 3' C3 propanediol spacer block
gctgtgattttggtctagctacagagaaatg

SEQ ID NO: 7 - DNA, 31 bp, Artificial Sequence
  Synthetic
  misc_feature (26)..(26): RNA
  misc_feature (31)..(31): 3' C3 propanediol spacer block
gccctcaattcttaccatccacaaaatggaa

SEQ ID NO: 8 - DNA, 401 bp, Artificial Sequence
  Synthetic
aaaaaataagaacactgatttttgtgaatactgggaactatgaaaatactatagttgagaccttcaatgactttctagtaactcagcagcatctcagggccaaaaatttaatcagtggaaaaatagcctcaattcttaccatccacaaaatggatccagacaactgttcaaactgatgggacccactccatcgagatttcactgtagctagaccaaaatcacctatttttactgtgaggtcttcatgaagaaatatatctgaggtgtagtaagtaaaggaaaacagtagatctcattttcctatcagagcaagcattatgaagagtttaggtaagagatctaatttctataattctgtaatataatattctttaaaacatagtacttcatctttcctctta

SEQ ID NO: 9 - DNA, 401 bp, Artificial Sequence
  Synthetic
aaaaaataagaacactgatttttgtgaatactgggaactatgaaaatactatagttgagaccttcaatgactttctagtaactcagcagcatctcagggccaaaaatttaatcagtggaaaaatagcctcaattcttaccatccacaaaatggatccagacaactgttcaaactgatgggacccactccatcgagatttctctgtagctagaccaaaatcacctatttttactgtgaggtcttcatgaagaaatatatctgaggtgtagtaagtaaaggaaaacagtagatctcattttcctatcagagcaagcattatgaagagtttaggtaagagatctaatttctataattctgtaatataatattctttaaaacatagtacttcatctttcctctta

SEQ ID NO: 10 - DNA, 29 bp, Artificial Sequence
  Synthetic
  misc_feature (26)..(26): RNA
  misc_feature (27)..(28): two C3 propanediol spacers
gctgtgattttggtctagctacagtgatg

SEQ ID NO: 11 - DNA, 29 bp, Artificial Sequence
  Synthetic
  misc_feature (26)..(26): RNA
  misc_feature (27)..(28): two C3 propanediol spacers
gctgtgattttggtctagctacagagatg

SEQ ID NO: 12 - DNA, 31 bp, Artificial Sequence; identical to SEQ ID NO: 7
  Synthetic
  misc_feature (26)..(26): RNA
  misc_feature (31)..(31): 3' C3 propanediol spacer

SEQ ID NO: 13 - DNA, 23 bp, Artificial Sequence
  Synthetic
cgccgcgtatagtcccgcgtaaa

SEQ ID NO: 14 - DNA, 13 bp, Artificial Sequence
  Synthetic
  misc_feature (1)..(1): 5' 6-carboxyfluorescein
  misc_feature (1)..(1): LNA residue
  misc_feature (5)..(7): LNA residues
  misc_feature (11)..(11): LNA residue
  misc_feature (13)..(13): 3' Iowa Black fluorescence quencher
ccatcaccgtgct

SEQ ID NO: 15 - DNA, 13 bp, Artificial Sequence
  Synthetic
  misc_feature (1)..(1): 5' 6-carboxy-2',4,4',5',7,7'-hexachlorofluorescein
  misc_feature (5)..(7): LNA residues
  misc_feature (11)..(11): LNA residue
  misc_feature (13)..(13): 3' Iowa Black fluorescence quencher
caatccccgagct

SEQ ID NO: 16 - DNA, 53 bp, Artificial Sequence
  Synthetic
  misc_feature (48)..(48): RNA
  misc_feature (53)..(53): 3' C3 propanediol spacer block
gcccatgtcccagcgaaccatcaccgtgctagccctcgatacagcccggccac

SEQ ID NO: 17 - DNA, 52 bp, Artificial Sequence
  Synthetic
  misc_feature (46)..(46): RNA
  misc_feature (52)..(52): 3' C3 propanediol spacer block
gcccatgtcccagcgaacaatccccgagctgccctcgatacagcctggccac

SEQ ID NO: 18 - DNA, 26 bp, Artificial Sequence
  Synthetic
  misc_feature (21)..(21): RNA
  misc_feature (26)..(26): 3' C3 propanediol spacer block
gcggccaggtatacggacatcatcca

SEQ ID NO: 19 - DNA, 401 bp, Artificial Sequence
  Synthetic
gttgggagctgggagggactgagttagggtgcacggggcggccagtctcaccactgaccagtttgtctgtctgtgtgtgtccatgtgcgagggcagaggaggaccccacatggaccgcagcagcgcccgaggccaggtatacggacatcatcctgtacgcgtcgggctccctggccttggctgtgctcctgctgctggccgggctgtatcgagggcaggcgctccacggccggcacccccgcccgcccgccactgtgcagaagctctcccgcttccctctggcccgacaggtactgggcgcatcccccacctcacatgtgacagcctgactccagcaggcagaaccaagtctcccactttgcagttctccctggagtcaggctcttccggcaagtcaagct

SEQ ID NO: 20 - DNA, 401 bp, Artificial Sequence
  Synthetic
gttgggagctgggagggactgagttagggtgcacggggcggccagtctcaccactgaccagtttgtctgtctgtgtgtgtccatgtgcgagggcagaggaggaccccacatggaccgcagcagcgcccgaggccaggtatacggacatcatcctgtacgcgtcgggctccctggccttggctgtgctcctgctgctggccaggctgtatcgagggcaggcgctccacggccggcacccccgcccgcccgccactgtgcagaagctctcccgcttccctctggcccgacaggtactgggcgcatcccccacctcacatgtgacagcctgactccagcaggcagaaccaagtctcccactttgcagttctccctggagtcaggctcttccggcaagtcaagct

SEQ ID NO: 21 - DNA, 19 bp, Artificial Sequence
  Synthetic
cggcccatgtcccagcgaa

SEQ ID NO: 22 - DNA, 13 bp, Artificial Sequence
  Synthetic
  misc_feature (1)..(1): 5' Yakima yellow
  misc_feature (1)..(1): LNA residue
  misc_feature (5)..(7): LNA residues
  misc_feature (11)..(11): LNA residue
  misc_feature (13)..(13): 3' Iowa Black fluorescence quencher
caatccccgagct

SEQ ID NO: 23 - DNA, 56 bp, Artificial Sequence
  Synthetic
  misc_feature (51)..(51): RNA
  misc_feature (56)..(56): 3' C3 propanediol spacer block
gcccatgtcccagcgaaccatcaccgtgctacttcccacaccctcatatcutgtta

SEQ ID NO: 24 - DNA, 59 bp, Artificial Sequence
  Synthetic
  misc_feature (54)..(54): RNA
  misc_feature (59)..(59): 3' C3 propanediol spacer block
gcccatgtcccagcgaacaatccccgagctcttacttcccacaccctcatatautgtta

SEQ ID NO: 25 - DNA, 32 bp, Artificial Sequence
  Synthetic
  misc_feature (27)..(27): RNA
  misc_feature (32)..(32): 3' C3 propanediol spacer block
gcgctaagtaaacattcctgattgcaacttat

SEQ ID NO: 26 - DNA, 490 bp, Artificial Sequence
  Synthetic
gattttttttttttggcatttcttcttagatttctatctcctaacataggatcacttatttgtgaaattatttgtataccttttttatggagtgatgatgtgatacaaattctatccttaaggatataagaacatcttttctttatattaggatttttctggacccatgagttacatgcttacttcccacaccctcatatcttgtttaaatttgtagaattaaattcataggtaattatttctgaaacttcttccctgtgtgagcaatctaaataattattacaatgccttaagttgcaatcaggaatgtttacttagcacagacttttttccccactactgcactcaaaggataacagatatatggcaaatctaaccatattctttgtcctttgtccatgttgcggagggaagctcatcagtggggccacgagctgagtgcgtcctgtcactccactcccatgtcccttgggaaggtctgagactaggg

SEQ ID NO: 27 - DNA, 490 bp, Artificial Sequence
  Synthetic
gattttttttttttggcatttcttcttagatttctatctcctaacataggatcacttatttgtgaaattatttgtataccttttttatggagtgatgatgtgatacaaattctatccttaaggatataagaacatcttttctttatattaggatttttctggacccatgagttacatgcttacttcccacaccctcatatattgtttaaatttgtagaattaaattcataggtaattatttctgaaacttcttccctgtgtgagcaatctaaataattattacaatgccttaagttgcaatcaggaatgtttacttagcacagacttttttccccactactgcactcaaaggataacagatatatggcaaatctaaccatattctttgtcctttgtccatgttgcggagggaagctcatcagtggggccacgagctgagtgcgtcctgtcactccactcccatgtcccttgggaaggtctgagactaggg

SEQ ID NO: 28 - DNA, 59 bp, Artificial Sequence
  Synthetic
  misc_feature (54)..(54): RNA
  misc_feature (59)..(59): 3' C3 propanediol spacer block
gcccatgtcccagcgaaccatcaccgtgctttctcttctggactccctataatattgtg

SEQ ID NO: 29 - DNA, 59 bp, Artificial Sequence
  Synthetic
  misc_feature (54)..(54): RNA
  misc_feature (59)..(59): 3' C3 propanediol spacer block
gcccatgtcccagcgaacaatccccgagctttctcttctggactccctataacattgtg

SEQ ID NO: 30 - DNA, 26 bp, Artificial Sequence
  Synthetic
  misc_feature (21)..(21): RNA
  misc_feature (26)..(26): 3' C3 propanediol spacer block
gcggattgatgcagcagtgagtcatg

SEQ ID NO: 31 - DNA, 56 bp, Artificial Sequence
  Synthetic
  misc_feature (51)..(51): RNA
  misc_feature (56)..(56): 3' C3 propanediol spacer block
gcccatgtcccagcgaaccatcaccgtgctctccgttgttttccagaaacgatttc

SEQ ID NO: 32 - DNA, 56 bp, Artificial Sequence
  Synthetic
  misc_feature (51)..(51): RNA
  misc_feature (56)..(56): 3' C3 propanediol spacer block
gcccatgtcccagcgaacaatccccgagctctccgttgttttccagaaatgatttc

SEQ ID NO: 33 - DNA, 56 bp, Artificial Sequence
  Synthetic
  misc_feature (51)..(51): RNA
  misc_feature (56)..(56): 3' C3 propanediol spacer block
gcccatgtcccagcgaacaatccccgagctctccgttgttttccagaaaggatttc

SEQ ID NO: 34 - DNA, 28 bp, Artificial Sequence
  Synthetic
  misc_feature (23)..(23): RNA
  misc_feature (28)..(28): 3' C3 propanediol spacer block
gcaaccaagtcttccctacaaccttgat

SEQ ID NO: 35 - DNA, 401 bp, Artificial Sequence
  Synthetic
acatcatttttattgtataaaagcattttagtatcaattttctcatttttaaaccaagtcttccctacaaccttgaataaatggtttccaaggaaaataaaatcttggccttacctggatccatggggagttcagaatcctgaagttttcattgaatcttttcatcagggtgagaaaattctgatctttataatcaaatcgtttctggaaaacaacggagcagatcacattgcagggagcacagcccaggatgaaagtgggatcacagggtgaagctaaagatttaaaaatttttaaaaaaattattaaaaaataaatatttaaaagatttgcatttgttaagacataaaggaaatttagaaattttaaacaatatcttacaaattccccatgtgtccaaa

SEQ ID NO: 36 - DNA, 401 bp, Artificial Sequence
  Synthetic
acatcatttttattgtataaaagcattttagtatcaattttctcatttttaaaccaagtcttccctacaaccttgaataaatggtttccaaggaaaataaaatcttggccttacctggatccatggggagttcagaatcctgaagttttcattgaatcttttcatcagggtgagaaaattctgatctttataatcaaatcatttctggaaaacaacggagcagatcacattgcagggagcacagcccaggatgaaagtgggatcacagggtgaagctaaagatttaaaaatttttaaaaaaattattaaaaaataaatatttaaaagatttgcatttgttaagacataaaggaaatttagaaattttaaacaatatcttacaaattccccatgtgtccaaa

SEQ ID NO: 37 - DNA, 401 bp, Artificial Sequence
  Synthetic
acatcatttttattgtataaaagcattttagtatcaattttctcatttttaaaccaagtcttccctacaaccttgaataaatggtttccaaggaaaataaaatcttggccttacctggatccatggggagttcagaatcctgaagttttcattgaatcttttcatcagggtgagaaaattctgatctttataatcaaatcctttctggaaaacaacggagcagatcacattgcagggagcacagcccaggatgaaagtgggatcacagggtgaagctaaagatttaaaaatttttaaaaaaattattaaaaaataaatatttaaaagatttgcatttgttaagacataaaggaaatttagaaattttaaacaatatcttacaaattccccatgtgtccaaa

SEQ ID NO: 38 - DNA, 56 bp, Artificial Sequence
  Synthetic
  misc_feature (51)..(51): RNA
  misc_feature (56)..(56): 3' C3 propanediol spacer block
gcccatgtcccagcgaaccatcaccgtgctgtctttgctttcctggtgagcccatg

SEQ ID NO: 39 - DNA, 55 bp, Artificial Sequence
  Synthetic
  misc_feature (49)..(49): RNA
  misc_feature (55)..(55): 3' C3 propanediol spacer block
gcccatgtcccagcgaacaatccccgagctgtctttgctttcctggtgacccatg

SEQ ID NO: 40 - DNA, 32 bp, Artificial Sequence
  Synthetic
  misc_feature (27)..(27): RNA
  misc_feature (32)..(32): 3' C3 propanediol spacer block
gcgttggaactaccacattgctttatugtact

SEQ ID NO: 41 - DNA, 19 bp, Artificial Sequence
  Synthetic
gcggagggaagctcatcag

SEQ ID NO: 42 - DNA, 22 bp, Artificial Sequence
  Synthetic
ccctagtctcagaccttcccaa

SEQ ID NO: 43 - DNA, 24 bp, Artificial Sequence
  Synthetic
  misc_feature (1)..(1): 5' Yakima yellow
  misc_feature (24)..(24): 3' Iowa Black fluorescence quencher
ccacgagctgagtgcgtcctgtca

SEQ ID NO: 44 - DNA, 50 bp, Artificial Sequence
  Synthetic
aatgatacggcgaccaccgagatctacactctttccctacacgacgctct

SEQ ID NO: 45 - DNA, 55 bp, Artificial Sequence
  Synthetic
caagcagaagacggcatacgagatggacctatgtgactggagttcagacgtgtgc

SEQ ID NO: 46 - DNA, 21 bp, Artificial Sequence
  Synthetic
  misc_feature (1)..(1): 5 universal domain (UniFor-UniPro-)
  misc_feature (16)..(16): RNA
  misc_feature (21)..(21): 3' propanediol (C3) spacer blocking group
ccctgggtccctgggagaatc

SEQ ID NO: 47 - DNA, 26 bp, Artificial Sequence
  GCK-356-2
  misc_feature (1)..(1): 5' universal domain (UniFor-UniPro-)
  misc_feature (21)..(21): RNA
  misc_feature (26)..(26): 3' propanediol (C3) spacer blocking group
cgaggagaaccacattctcccagggt

SEQ ID NO: 48 - DNA, 18 bp, Artificial Sequence
  ERBB3-33-1
  misc_feature (1)..(1): 5 universal domain (UniFor-UniPro-)
  misc_feature (14)..(14): RNA
  misc_feature (18)..(18): 3' propanediol (C3) spacer blocking group
gggcggccgtgacucacc

SEQ ID NO: 49 - DNA, 24 bp, Artificial Sequence
  ERBB3-33-2
  misc_feature (1)..(1): 5 universal domain (UniFor-UniPro-)
  misc_feature (18)..(18): RNA
  misc_feature (24)..(24): 3' propanediol (C3) spacer blocking group
gagggaagggggtgagtcacggcg

SEQ ID NO: 50 - DNA, 25 bp, Artificial Sequence
  TTR-1257-1
  misc_feature (1)..(1): 5' universal domain (UniFor-UniPro-)
  misc_feature (20)..(20): RNA
  misc_feature (25)..(25): 3' propanediol (C3) spacer blocking group
cctgggagccatttgcctcugggtt

SEQ ID NO: 51 - DNA, 27 bp, Artificial Sequence
  TTR-1257-2
  misc_feature (1)..(1): 5' universal domain (UniFor-UniPro-)
  misc_feature (22)..(22): RNA
  misc_feature (27)..(27): 3' propanediol (C3) spacer blocking group
ctttggcaacttacccagaggcaaatc

SEQ ID NO: 52 - DNA, 22 bp, Artificial Sequence
  HAMP-253-1
  misc_feature (1)..(1): 5' universal domain (UniFor-UniPro-)
  misc_feature (17)..(17): RNA
  misc_feature (22)..(22): 3' propanediol (C3) spacer blocking group
gcactgagctcccagauctggc

SEQ ID NO: 53 - DNA, 22 bp, Artificial Sequence
  HAMP-253-2
  misc_feature (1)..(1): 5' universal domain (UniFor-UniPro-)
  misc_feature (17)..(17): RNA
  misc_feature (22)..(22): 3' propanediol (C3) spacer blocking group
gcaagcggcccagatcugggac

SEQ ID NO: 54 - DNA, 27 bp, Artificial Sequence
  BIRC5-606-1
  misc_feature (1)..(1): 5' universal domain (UniFor-UniPro-)
  misc_feature (22)..(22): RNA
  misc_feature (27)..(27): 3' propanediol (C3) spacer blocking group
gacgaccccatgtaagtcttcuctggg

SEQ ID NO: 55 - DNA, 23 bp, Artificial Sequence
  BIRC5-606-2
  misc_feature (1)..(1): 5' universal domain (UniFor-UniPro-)
  misc_feature (17)..(17): RNA
  misc_feature (23)..(23): 3' propanediol (C3) spacer blocking group
cgaggctggccagagaagacttt

SEQ ID NO: 56 - DNA, 36 bp, Artificial Sequence
  SAA 146-1
  misc_feature (1)..(1): 5' universal domain (UniFor-UniPro-)
  misc_feature (31)..(31): RNA
  misc_feature (36)..(36): 3' propanediol (C3) spacer blocking group
ctttcccaacaagattatcatttcctttaaaaaaat

SEQ ID NO: 57 - DNA, 30 bp, Artificial Sequence
  SAA 146-2
  misc_feature (1)..(1): 5' universal domain (UniFor-UniPro-)
  misc_feature (25)..(25): RNA
  misc_feature (30)..(30): 3' propanediol (C3) spacer blocking group
cgccccaggataactattttttttaaaggt

SEQ ID NO: 58 - DNA, 23 bp, Artificial Sequence
  IDO1-97-1
  misc_feature (1)..(1): 5' universal domain (UniFor-UniPro-)
  misc_feature (18)..(18): RNA
  misc_feature (23)..(23): 3' propanediol (C3) spacer blocking group
agacactgaggggcaccagaggt

SEQ ID NO: 59 - DNA, 26 bp, Artificial Sequence
  IDO1-97-2
  misc_feature (1)..(1): 5' universal domain (UniFor-UniPro-)
  misc_feature (21)..(21): RNA
  misc_feature (26)..(26): 3' propanediol (C3) spacer blocking group
cttgtagtctgctcctctggugcccg

SEQ ID NO: 60 - DNA, 33 bp, Artificial Sequence
  IDO1-176-1
  misc_feature (1)..(1): 5' universal domain (UniFor-UniPro-)
  misc_feature (28)..(28): RNA
  misc_feature (33)..(33): 3' propanediol (C3) spacer blocking group
agtaaagagtaccatattgatgaagaagtggga

SEQ ID NO: 61 - DNA, 24 bp, Artificial Sequence
  IDO1-176-2
  misc_feature (1)..(1): 5' universal domain (UniFor-UniPro-)
  misc_feature (19)..(19): RNA
  misc_feature (24)..(24): 3' propanediol (C3) spacer blocking group
gcagagcaaagcccacttcttcaa

SEQ ID NO: 62 - DNA, 25 bp, Artificial Sequence
  CYP27A-31016-1
  misc_feature (1)..(1): 5' universal domain (UniFor-UniPro-)
  misc_feature (20)..(20): RNA
  misc_feature (25)..(25): 3' propanediol (C3) spacer blocking group
cctttggtgaggactcccagatggc

SEQ ID NO: 63 - DNA, 21 bp, Artificial Sequence
  CYP27A-31016-2
  misc_feature (1)..(1): 5' universal domain (UniFor-UniPro-)
  misc_feature (16)..(16): RNA
  misc_feature (21)..(21): 3' propanediol (C3) spacer blocking group
cctgggccccatctgggagtg

SEQ ID NO: 64 - DNA, 30 bp, Artificial Sequence
  SAA 226-1
  misc_feature (1)..(1): 5' universal domain (UniFor-UniPro-)
  misc_feature (25)..(25): RNA
  misc_feature (30)..(30): 3' propanediol (C3) spacer blocking group
tctcctctgatctagagaggtaagcaggga

SEQ ID NO: 65 - DNA, 24 bp, Artificial Sequence
  SAA 226-2
  misc_feature (1)..(1): 5' universal domain (UniFor-UniPro-)
  misc_feature (19)..(19): RNA
  misc_feature (24)..(24): 3' propanediol (C3) spacer blocking group
accaggcccgaccctgctuacctg

SEQ ID NO: 66 - DNA, 26 bp, Artificial Sequence
  KIF11-369-1
  misc_feature (1)..(1): 5' universal domain (UniFor-UniPro-)
  misc_feature (21)..(21): RNA
  misc_feature (26)..(26): 3' propanediol (C3) spacer blocking group
gagaaggggaagaacatccaggtgga

SEQ ID NO: 67 - DNA, 24 bp, Artificial Sequence
  KIF11-369-2
  misc_feature (1)..(1): 5' universal domain (UniFor-UniPro-)
  misc_feature (19)..(19): RNA
  misc_feature (24)..(24): 3' propanediol (C3) spacer blocking group
gcatctcaccaccacctggatgta

SEQ ID NO: 68 - DNA, 28 bp, Artificial Sequence
  C3-1394-1
  misc_feature (1)..(1): 5' universal domain (UniFor-UniPro-)
  misc_feature (23)..(23): RNA
  misc_feature (28)..(28): 3' propanediol (C3) spacer blocking group
ctggacagcactagttttttgcctgggt

SEQ ID NO: 69 - DNA, 22 bp, Artificial Sequence
  C3-1394-2
  misc_feature (1)..(1): 5' universal domain (UniFor-UniPro-)
  misc_feature (17)..(17): RNA
  misc_feature (22)..(22): 3' propanediol (C3) spacer blocking group
ccacgacttcccaggcaaaaat

SEQ ID NO: 70 - DNA, 23 bp, Artificial Sequence
  HOGA-505-1
  misc_feature (1)..(1): 5' universal domain (UniFor-UniPro-)
  misc_feature (18)..(18): RNA
  misc_feature (23)..(23): 3' propanediol (C3) spacer blocking group
cactgcagaggtggactatgggt

SEQ ID NO: 71 - DNA, 29 bp, Artificial Sequence
  HOGA-505-2
  misc_feature (1)..(1): 5' universal domain (UniFor-UniPro-)
  misc_feature (24)..(24): RNA
  misc_feature (29)..(29): 3' propanediol (C3) spacer blocking group
gattctcctccagtttcccataguccacg

SEQ ID NO: 72 - DNA, 30 bp, Artificial Sequence
  EGFR-123344-1
  misc_feature (1)..(1): 5' universal domain (UniFor-UniPro-)
  misc_feature (25)..(25): RNA
  misc_feature (30)..(30): 3' propanediol (C3) spacer blocking group
ccagaggatgttcaataactgtgaggtgga

SEQ ID NO: 73 - DNA, 25 bp, Artificial Sequence
  EGFR-123344-2
  misc_feature (1)..(1): 5' universal domain (UniFor-UniPro-)
  misc_feature (20)..(20): RNA
  misc_feature (25)..(25): 3' propanediol (C3) spacer blocking group
caaattcccaaggaccaccucacac

SEQ ID NO: 74 - DNA, 25 bp, Artificial Sequence
  ALDH2-15144-1
  misc_feature (1)..(1): 5' universal domain (UniFor-UniPro-)
  misc_feature (20)..(20): RNA
  misc_feature (25)..(25): 3' propanediol (C3) spacer blocking group
tgaaggggacaaggtgagaactgga

SEQ ID NO: 75 - DNA, 27 bp, Artificial Sequence
  ALDH2-15144-2
  misc_feature (1)..(1): 5' universal domain (UniFor-UniPro-)
  misc_feature (22)..(22): RNA
  misc_feature (27)..(27): 3' propanediol (C3) spacer blocking group
cccaaggtaagtcaccagttcucacca

SEQ ID NO: 76 - DNA, 25 bp, Artificial Sequence
  AGXT-140-1
  misc_feature (1)..(1): 5' universal domain (UniFor-UniPro-)
  misc_feature (20)..(20): RNA
  misc_feature (25)..(25): 3' propanediol (C3) spacer blocking group
ccatggcctctcacaagctgctgga

SEQ ID NO: 77 - DNA, 21 bp, Artificial Sequence
  AGXT-140-2
  misc_feature (1)..(1): 5' universal domain (UniFor-UniPro-)
  misc_feature (16)..(16): RNA
  misc_feature (21)..(21): 3' propanediol (C3) spacer blocking group
gggggtcaccagcagcttgtc

SEQ ID NO: 78 - DNA, 30 bp, Artificial Sequence
  APOC-2929-1
  misc_feature (1)..(1): 5' universal domain (UniFor-UniPro-)
  misc_feature (25)..(25): RNA
  misc_feature (30)..(30): 3' propanediol (C3) spacer blocking group
ccgttaaggacaagttctctgagtuctggc

SEQ ID NO: 79 - DNA, 27 bp, Artificial Sequence
  APOC-2929-2
  misc_feature (1)..(1): 5' universal domain (UniFor-UniPro-)
  misc_feature (22)..(22): RNA
  misc_feature (27)..(27): 3' propanediol (C3) spacer blocking group
tcagggtccaaatcccagaacucagac

SEQ ID NO: 80 - DNA, 36 bp, Artificial Sequence
  Met 27554-1
  misc_feature (1)..(1): 5' universal domain (UniFor-UniPro-)
  misc_feature (31)..(31): RNA
  misc_feature (36)..(36): 3' propanediol (C3) spacer blocking group
aattttatttacttcttgacggtccaaagggaaaca

SEQ ID NO: 81 - DNA, 28 bp, Artificial Sequence
  Met 27554-2
  misc_feature (1)..(1): 5' universal domain (UniFor-UniPro-)
  misc_feature (23)..(23): RNA
  misc_feature (28)..(28): 3' propanediol (C3) spacer blocking group
gtctgagcatctagagtttcccuttggt

SEQ ID NO: 82 - DNA, 27 bp, Artificial Sequence
  SAA 88-1
  misc_feature (1)..(1): 5' universal domain (UniFor-UniPro-)
  misc_feature (22)..(22): RNA
  misc_feature (27)..(27): 3' propanediol (C3) spacer blocking group
aggtgaggagcacaccaaggagtgata

SEQ ID NO: 83 - DNA, 35 bp, Artificial Sequence
  SAA 88-2
  misc_feature (1)..(1): 5' universal domain (UniFor-UniPro-)
  misc_feature (30)..(30): RNA
  misc_feature (35)..(35): 3' propanediol (C3) spacer blocking group
gaaaacagagtaagttttaaaaatcactccttgga

SEQ ID NO: 84 - DNA, 20 bp, Artificial Sequence
  HIF1A-293-1
  misc_feature (1)..(1): 5' universal domain (UniFor-UniPro-)
  misc_feature (15)..(15): RNA
  misc_feature (20)..(20): 3' propanediol (C3) spacer blocking group
tcgcacccccacctctggag

SEQ ID NO: 85 - DNA, 27 bp, Artificial Sequence
  HIF1A-293-2
  misc_feature (1)..(1): 5' universal domain (UniFor-UniPro-)
  misc_feature (22)..(22): RNA
  misc_feature (27)..(27): 3' propanediol (C3) spacer blocking group
gaaggaaaggcaagtccagaggtgggc

SEQ ID NO: 86 - DNA, 36 bp, Artificial Sequence; identical to SEQ ID NO: 80
  Met 27475-1
  misc_feature (1)..(1): 5' universal domain (UniFor-UniPro-)
  misc_feature (31)..(31): RNA
  misc_feature (36)..(36): 3' propanediol (C3) spacer blocking group

SEQ ID NO: 87 - DNA, 28 bp, Artificial Sequence
  Met 27475-2
  misc_feature (1)..(1): 5' universal domain (UniFor-UniPro-)
  misc_feature (23)..(23): RNA
  misc_feature (28)..(28): 3' propanediol (C3) spacer blocking group
gtctgagcatctagagtttcccuttggt

SEQ ID NO: 88 - DNA, 21 bp, Artificial Sequence
  HAMP-295-1
  misc_feature (1)..(1): 5' universal domain (UniFor-UniPro-)
  misc_feature (16)..(16): RNA
  misc_feature (21)..(21): 3' propanediol (C3) spacer blocking group
ctcgccagcctgaccagtggg

SEQ ID NO: 89 - DNA, 25 bp, Artificial Sequence
  HAMP-295-2
  misc_feature (1)..(1): 5' universal domain (UniFor-UniPro-)
  misc_feature (20)..(20): RNA
  misc_feature (25)..(25): 3' propanediol (C3) spacer blocking group
gggaaaacagagccactggucaggg

SEQ ID NO: 90 - DNA, 22 bp, Artificial Sequence
  GRHPR-2234-1
  misc_feature (1)..(1): 5' universal domain (UniFor-UniPro-)
  misc_feature (17)..(17): RNA
  misc_feature (22)..(22): 3' propanediol (C3) spacer blocking group
gcctcctctccgaccacgtggt

SEQ ID NO: 91 - DNA, 26 bp, Artificial Sequence
  GRHPR-2234-2
  misc_feature (1)..(1): 5' universal domain (UniFor-UniPro-)
  misc_feature (20)..(20): RNA
  misc_feature (26)..(26): 3' propanediol (C3) spacer blocking group
ggatcctcttgtccacgtggtcggac

SEQ ID NO: 92 - DNA, 20 bp, Artificial Sequence
  HAMP-88-1
  misc_feature (1)..(1): 5' universal domain (UniFor-UniPro-)
  misc_feature (15)..(15): RNA
  misc_feature (20)..(20): 3' propanediol (C3) spacer blocking group
ggcgccaccaccttcttggt

SEQ ID NO: 93 - DNA, 27 bp, Artificial Sequence
  HAMP-88-2
  misc_feature (1)..(1): 5' universal domain (UniFor-UniPro-)
  misc_feature (22)..(22): RNA
  misc_feature (27)..(27): 3' propanediol (C3) spacer blocking group
gctctgtctcatttccaagaaggtgga

SEQ ID NO: 94 - DNA, 28 bp, Artificial Sequence
  Met 27254-1
  misc_feature (1)..(1): 5' universal domain (UniFor-UniPro-)
  misc_feature (23)..(23): RNA
  misc_feature (28)..(28): 3' propanediol (C3) spacer blocking group
gagccaaagtcctttcatctgtaaaggt

SEQ ID NO: 95 - DNA, 30 bp, Artificial Sequence
  Met 27254-2
  misc_feature (1)..(1): 5' universal domain (UniFor-UniPro-)
  misc_feature (25)..(25): RNA
  misc_feature (30)..(30): 3' propanediol (C3) spacer blocking group
gaagttgatgaaccggtcctttacagatgt

SEQ ID NO: 96 - DNA, 26 bp, Artificial Sequence
  GRHPR-2264-1
  misc_feature (1)..(1): 5' universal domain (UniFor-UniPro-)
  misc_feature (21)..(21): RNA
  misc_feature (26)..(26): 3' propanediol (C3) spacer blocking group
acaagaggatcctggatgctgcagga

SEQ ID NO: 97 - DNA, 23 bp, Artificial Sequence
  GRHPR-2264-2
  misc_feature (1)..(1): 5' universal domain (UniFor-UniPro-)
  misc_feature (18)..(18): RNA
  misc_feature (23)..(23): 3' propanediol (C3) spacer blocking group
cgctctagctccttggcagggaa

SEQ ID NO: 98 - DNA, 27 bp, Artificial Sequence
  Serpina 279-1
  misc_feature (1)..(1): 5' universal domain (UniFor-UniPro-)
  misc_feature (22)..(22): RNA
  misc_feature (27)..(27): 3' propanediol (C3) spacer blocking group
actcagttccacaggtgggagggaggc

SEQ ID NO: 99 - DNA, 27 bp, Artificial Sequence
  Serpina 279-2
  misc_feature (1)..(1): 5' universal domain (UniFor-UniPro-)
  misc_feature (22)..(22): RNA
  misc_feature (27)..(27): 3' propanediol (C3) spacer blocking group
cactctaagccctgctgtcccacctga

SEQ ID NO: 100 - DNA, 27 bp, Artificial Sequence
  Myc 459-1
  misc_feature (1)..(1): 5' universal domain (UniFor-UniPro-)
  misc_feature (22)..(22): RNA
  misc_feature (27)..(27): 3' propanediol (C3) spacer blocking group
cgggaggctattctgcccattugggat

SEQ ID NO: 101 - DNA, 24 bp, Artificial Sequence
  Myc 459-2
  misc_feature (1)..(1): 5' universal domain (UniFor-UniPro-)
  misc_feature (19)..(19): RNA
  misc_feature (24)..(24): 3' propanediol (C3) spacer blocking group
cggggaagtgtccccaaaugggct

SEQ ID NO: 102 - DNA, 23 bp, Artificial Sequence
  Serpina 130-1
  misc_feature (1)..(1): 5' universal domain (UniFor-UniPro-)
  misc_feature (18)..(18): RNA
  misc_feature (23)..(23): 3' propanediol (C3) spacer blocking group
gctgctgctgccaggaautccac

SEQ ID NO: 103 - DNA, 24 bp, Artificial Sequence
  Serpina 130-2
  misc_feature (1)..(1): 5' universal domain (UniFor-UniPro-)
  misc_feature (19)..(19): RNA
  misc_feature (24)..(24): 3' propanediol (C3) spacer blocking group
cccctccaacctggaattcctggg

SEQ ID NO: 104 - DNA, 23 bp, Artificial Sequence
  Myc 490-1
  misc_feature (1)..(1): 5' universal domain (UniFor-UniPro-)
  misc_feature (18)..(18): RNA
  misc_feature (23)..(23): 3' propanediol (C3) spacer blocking group
ctgccaggacccgcttcuctgat

SEQ ID NO: 105 - DNA, 26 bp, Artificial Sequence
  Myc 490-2
  misc_feature (1)..(1): 5' universal domain (UniFor-UniPro-)
  misc_feature (21)..(21): RNA
  misc_feature (26)..(26): 3' propanediol (C3) spacer blocking group
caaggagagcctttcagagaagcggc

SEQ ID NO: 106 - DNA, 23 bp, Artificial Sequence
  GRHPR-2179-1
  misc_feature (1)..(1): 5' universal domain (UniFor-UniPro-)
  misc_feature (18)..(18): RNA
  misc_feature (23)..(23): 3' propanediol (C3) spacer blocking group
gatgagcccatccctgccaaggt

SEQ ID NO: 107 - DNA, 23 bp, Artificial Sequence
  GRHPR-2179-2
  misc_feature (1)..(1): 5' universal domain (UniFor-UniPro-)
  misc_feature (18)..(18): RNA
  misc_feature (23)..(23): 3' propanediol (C3) spacer blocking group
cgctctagctccttggcagggaa

SEQ ID NO: 108 - DNA, 21 bp, Artificial Sequence
  GYG-2851-1
  misc_feature (1)..(1): 5' universal domain (UniFor-UniPro-)
  misc_feature (16)..(16): RNA
  misc_feature (21)..(21): 3' propanediol (C3) spacer blocking group
tcgccacccctcagguctcac

SEQ ID NO: 109 - DNA, 26 bp, Artificial Sequence
  GYG-2851-2
  misc_feature (1)..(1): 5' universal domain (UniFor-UniPro-)
  misc_feature (21)..(21): RNA
  misc_feature (26)..(26): 3' propanediol (C3) spacer blocking group
acctcatggagtctgagaccugaggc

SEQ ID NO: 110 - DNA, 21 bp, Artificial Sequence
  GYG-2793-1
  misc_feature (1)..(1): 5' universal domain (UniFor-UniPro-)
  misc_feature (16)..(16): RNA
  misc_feature (21)..(21): 3' propanediol (C3) spacer blocking group
gccctggtcctgggaucatca

SEQ ID NO: 111 - DNA, 28 bp, Artificial Sequence
  GYG-2793-2
  misc_feature (1)..(1): 5' universal domain (UniFor-UniPro-)
  misc_feature (23)..(23): RNA
  misc_feature (28)..(28): 3' propanediol (C3) spacer blocking group
ctgtgctgtttcagagatgatcccaggt

SEQ ID NO: 112 - DNA, 28 bp, Artificial Sequence
  Serpina 79-1
  misc_feature (1)..(1): 5' universal domain (UniFor-UniPro-)
  misc_feature (23)..(23): RNA
  misc_feature (28)..(28): 3' propanediol (C3) spacer blocking group
caagagtcctgagctgaaccaagaaggt

SEQ ID NO: 113 - DNA, 25 bp, Artificial Sequence
  Serpina 79-2
  misc_feature (1)..(1): 5' universal domain (UniFor-UniPro-)
  misc_feature (20)..(20): RNA
  misc_feature (25)..(25): 3' propanediol (C3) spacer blocking group
cgaccccctcctccttcttggttct

SEQ ID NO: 114 - DNA, 28 bp, Artificial Sequence
  Myc 538-1
  misc_feature (1)..(1): 5' universal domain (UniFor-UniPro-)
  misc_feature (23)..(23): RNA
  misc_feature (28)..(28): 3' propanediol (C3) spacer blocking group
ctgcttagacgctggattttttucggga

SEQ ID NO: 115 - DNA, 27 bp, Artificial Sequence
  Myc 538-2
  misc_feature (1)..(1): 5' universal domain (UniFor-UniPro-)
  misc_feature (22)..(22): RNA
  misc_feature (27)..(27): 3' propanediol (C3) spacer blocking group
ctggttttccactacccgaaaraaaaa

SEQ ID NO: 116 - DNA, 31 bp, Artificial Sequence
  GYG-2744-1
  misc_feature (1)..(1): 5' universal domain (UniFor-UniPro-)
  misc_feature (26)..(26): RNA
  misc_feature (31)..(31): 3' propanediol (C3) spacer blocking group
ctttgtattaagatcaggcctttgtgacaca

SEQ ID NO: 117 - DNA, 28 bp, Artificial Sequence
  GYG-2744-2
  misc_feature (1)..(1): 5' universal domain (UniFor-UniPro-)
  misc_feature (23)..(23): RNA
  misc_feature (28)..(28): 3' propanediol (C3) spacer blocking group
catcgtttgtggttagtgtcacaaaggg

SEQ ID NO: 118 - DNA, 19 bp, Artificial Sequence
  RNase P For
gcggagggaagctcatcag

SEQ ID NO: 119 - DNA, 22 bp, Artificial Sequence
  RNase P Rev
ccctagtctcagaccttcccaa

SEQ ID NO: 120 - DNA, 24 bp, Artificial Sequence
  RNase P probe
  misc_feature (1)..(1): 5' 6-Fluorescein fluorescent dye (FAM)
  misc_feature (24)..(24): 3' Iowa Black fluorescent quencher (IBFQ)
ccacgagctgagtgcgtcctgtca

SEQ ID NO: 121 - DNA, 22 bp, Artificial Sequence
  GCK-356-1
gaggaaactgtgactgaacctc

SEQ ID NO: 122 - DNA, 16 bp, Artificial Sequence
  GCK-356-2
ccaaggcttctccgcc

SEQ ID NO: 123 - DNA, 17 bp, Artificial Sequence
  ERBB3-33-1
gagtccggggagggatg

SEQ ID NO: 124 - DNA, 19 bp, Artificial Sequence
  ERBB3-33-2
caatccctactccagcctc

SEQ ID NO: 125 - DNA, 21 bp, Artificial Sequence
  TTR-1257-1
atgtgagcctctctctaccaa

SEQ ID NO: 126 - DNA, 23 bp, Artificial Sequence
  TTR-1257-2
gtcctctgatggtcaaagttcta

SEQ ID NO: 127 - DNA, 16 bp, Artificial Sequence
  HAMP-253-1
cactggtcaggctggc

SEQ ID NO: 128 - DNA, 18 bp, Artificial Sequence
  HAMP-253-2
caagctcaagacccagca

SEQ ID NO: 129 - DNA, 25 bp, Artificial Sequence
  BIRC5-606-1
caactcaaatcttttgacaactcag

SEQ ID NO: 130 - DNA, 16 bp, Artificial Sequence
  BIRC5-606-2
ggagctggaaggctgg

SEQ ID NO: 131 - DNA, 23 bp, Artificial Sequence
  SAA 146-1
ttcagaatggtatggctgtatgc

SEQ ID NO: 132 - DNA, 20 bp, Artificial Sequence
  SAA 146-2
cacagatcaggtgaggagca

SEQ ID NO: 133 - DNA, 19 bp, Artificial Sequence
  IDO1-97-1
gttttccatagcgtgtgcc

SEQ ID NO: 134 - DNA, 17 bp, Artificial Sequence
  IDO1-97-2
gtggtcactggctgtgg

SEQ ID NO: 135 - DNA, 23 bp, Artificial Sequence
  IDO1-176-1
ttcccacattttactgccttctc

SEQ ID NO: 136 - DNA, 20 bp, Artificial Sequence
  IDO1-176-2
cgctatggaaaactcctgga

SEQ ID NO: 137 - DNA, 18 bp, Artificial Sequence
  CYP27A-31016-1
caggtctgtgcatcagcg

SEQ ID NO: 138 - DNA, 20 bp, Artificial Sequence
  CYP27A-31016-2
ctttctggaagcgatacctg

SEQ ID NO: 139 - DNA, 20 bp, Artificial Sequence
  SAA 226-1
cgcacagaactcaacatggg

SEQ ID NO: 140 - DNA, 24 bp, Artificial Sequence
  SAA 226-2
aatagttatcctggggcatacagc

SEQ ID NO: 141 - DNA, 18 bp, Artificial Sequence
  KIF11-369-1
gctcggaatcctgtcagc

SEQ ID NO: 142 - DNA, 18 bp, Artificial Sequence
  KIF11-369-2
cagccaaattcgtctgcg

SEQ ID NO: 143 - DNA, 22 bp, Artificial Sequence
  C3-1394-1
gggatgttccagtcactgttac

SEQ ID NO: 144 - DNA, 15 bp, Artificial Sequence
  C3-1394-2
ggttggtggcagggg

SEQ ID NO: 145 - DNA, 16 bp, Artificial Sequence
  HOGA-505-1
aggggaaggtgcccag

SEQ ID NO: 146 - DNA, 17 bp, Artificial Sequence
  HOGA-505-2
aaggtggacattgcggg

SEQ ID NO: 147 - DNA, 23 bp, Artificial Sequence
  EGFR-123344-1
tcataattcctctgcacataggt

SEQ ID NO: 148 - DNA, 18 bp, Artificial Sequence
  EGFR-123344-2
gccaaggcacgagtaaca

SEQ ID NO: 149 - DNA, 28 bp, Artificial Sequence
  ALDH2-15144-1
cgtataaaatagaagacgaatccatccc

SEQ ID NO: 150 - DNA, 15 bp, Artificial Sequence
  ALDH2-15144-2
atggcacgatgccgt

SEQ ID NO: 151 - DNA, 15 bp, Artificial Sequence
  AGXT-140-1
ggcttgagcagggcc

SEQ ID NO: 152 - DNA, 15 bp, Artificial Sequence
  AGXT-140-2
tggccaaggccagtg

SEQ ID NO: 153 - DNA, 15 bp, Artificial Sequence
  APOC-2929-1
tcaggcagccacggc

SEQ ID NO: 154 - DNA, 18 bp, Artificial Sequence
  APOC-2929-2
gtgaccgatggcttcagt

SEQ ID NO: 155 - DNA, 27 bp, Artificial Sequence
  Met 27554-1
catacgcagcctgaagtatattaaaca

SEQ ID NO: 156 - DNA, 26 bp, Artificial Sequence
  Met 27554-2
tagatgctcagacttttcacacaaga

SEQ ID NO: 157 - DNA, 23 bp, Artificial Sequence
  SAA 88-1
ttcagaatggtatggctgtatgc

SEQ ID NO: 158 - DNA, 25 bp, Artificial Sequence
  SAA 88-2
agcagggaaggctcagtataaatag

SEQ ID NO: 159 - DNA, 16 bp, Artificial Sequence
  HIF1A-293-1
taagcgctggctccct

SEQ ID NO: 160 - DNA, 20 bp, Artificial Sequence
  HIF1A-293-2
ctctagtctcacgaggggtt

SEQ ID NO: 161 - DNA, 26 bp, Artificial Sequence
  Met 27475-1
ctcttttctgtgagaatacactccag

SEQ ID NO: 162 - DNA, 24 bp, Artificial Sequence
  Met 27475-2
taccccattaagtatgtccatgcc

SEQ ID NO: 163 - DNA, 17 bp, Artificial Sequence
  HAMP-295-1
tctcccatccctgctgc

SEQ ID NO: 164 - DNA, 15 bp, Artificial Sequence
  HAMP-295-2
ccgcttgcctcctgc

SEQ ID NO: 165 - DNA, 16 bp, Artificial Sequence
  GRHPR-2234-1
cacccagtgtgcacct

SEQ ID NO: 166 - DNA, 18 bp, Artificial Sequence
  GRHPR-2234-2
gccaaggagctagagcga

SEQ ID NO: 167 - DNA, 16 bp, Artificial Sequence
  HAMP-88-1
gaggcggtggtctgag

SEQ ID NO: 168 - DNA, 17 bp, Artificial Sequence
  HAMP-88-2
tgttccctgtcgctctg

SEQ ID NO: 169 - DNA, 27 bp, Artificial Sequence
  Met 27254-1
ctttagccttctcactgatatcgaatg

SEQ ID NO: 170 - DNA, 25 bp, Artificial Sequence
  Met 27254-2
gcatattctccccacagatagaaga

SEQ ID NO: 171 - DNA, 15 bp, Artificial Sequence
  GRHPR-2264-1
cctgcccacccagtg

SEQ ID NO: 172 - DNA, 18 bp, Artificial Sequence
  GRHPR-2264-2
ctgtgaggtggagcagtg

SEQ ID NO: 173 - DNA, 21 bp, Artificial Sequence
  Serpina 279-1
tagctcctgggcatttcttcc

SEQ ID NO: 174 - DNA, 21 bp, Artificial Sequence
  Serpina 279-2
agcttgaggagagcaggaaag

SEQ ID NO: 175 - DNA, 20 bp, Artificial Sequence
  Myc 459-1
cctggttttccactacccga

SEQ ID NO: 176 - DNA, 21 bp, Artificial Sequence
  Myc 459-2
cactggaacttacaacacccg

SEQ ID NO: 177 - DNA, 21 bp, Artificial Sequence
  Serpina 130-1
ttcctgctctcctcaagctct

SEQ ID NO: 178 - DNA, 21 bp, Artificial Sequence
  Serpina 130-2
gagctgaaccaagaaggagga

SEQ ID NO: 179 - DNA, 21 bp, Artificial Sequence
  Myc 490-1
aggcattcgactcatctcagc

SEQ ID NO: 180 - DNA, 21 bp, Artificial Sequence
  Myc 490-2
tgcactggaacttacaacacc

SEQ ID NO: 181 - DNA, 17 bp, Artificial Sequence
  GRHPR-2179-1
tcggagaggaggcagag

SEQ ID NO: 182 - DNA, 17 bp, Artificial Sequence
  GRHPR-2179-2
ttctcctgagggcctcc

SEQ ID NO: 183 - DNA, 21 bp, Artificial Sequence
  GYG-2851-1
acagggagaaggatgtcagag

SEQ ID NO: 184 - DNA, 22 bp, Artificial Sequence
  GYG-2851-2
gtcctgggatcatctctgaaac

SEQ ID NO: 185 - DNA, 21 bp, Artificial Sequence
  GYG-2793-1
acagggagaaggatgtcagag

SEQ ID NO: 186 - DNA, 21 bp, Artificial Sequence
  GYG-2793-2
cactaaccacaaacgatgcct

SEQ ID NO: 187 - DNA, 18 bp, Artificial Sequence
  Serpina 79-1
gaattcctggcagcagca

SEQ ID NO: 188 - DNA, 18 bp, Artificial Sequence
  Serpina 79-2
ctactgcctccacccgaa

SEQ ID NO: 189 - DNA, 22 bp, Artificial Sequence
  Myc 538-1
taggcattcgactcatctcagc

SEQ ID NO: 190 - DNA, 21 bp, Artificial Sequence
  Myc 538-2
tgcactggaacttacaacacc

SEQ ID NO: 191 - DNA, 17 bp, Artificial Sequence
  GYG-2744-1
ggaccagggcacctttg

SEQ ID NO: 192 - DNA, 23 bp, Artificial Sequence
  GYG-2744-2
ggctttctccagataagatactg

SEQ ID NO: 193 - DNA, 53 bp, Artificial Sequence
  Synthetic
tgcaggtgcagatgaagctggtcgtgccccagttattggtccgctggttattg

SEQ ID NO: 194 - DNA, 53 bp, Artificial Sequence
  Synthetic
caataaccagcggaccaataactggggcacgaccagcttcatctgcacctgca

SEQ ID NO: 195 - DNA, 53 bp, Artificial Sequence
  Synthetic
aggtgcagatgaagctggtcgtggtacggttattggtccgctggttattgttg

SEQ ID NO: 196 - DNA, 53 bp, Artificial Sequence
  Synthetic
caacaataaccagcggaccaataaccgtaccacgaccagcttcatctgcacct

SEQ ID NO: 197 - protein, 224 aa, Pyrococcus abyssi
MKVAGADEAGRGPVIGPLVIVAAVVEEDKIRSLTKLGVKDSKQLTPAQREKLFDEIVKVLDDYSVVIVSPQDIDGRKGSMNELEVENFVKALNSLKVKPEVIYIDSADVKAERFAENIRSRLAYEAKVVAEHKADAKYEIVSAASILAKVIRDREIEKLKAEYGDFGSGYPSDPRTKKWLEEWYSKHGNFPPIVRRTWDTAKKIEEKFKRAQLTLDNFLKRFRN

SEQ ID NO: 198 - protein, 224 aa, Artificial Sequence
  Synthetic
MKVAGADEAGRAPVIGPLVIVAAVVEEDKIRSLTKLGVKDSKQLTPAQREKLFDEIVKVLDDYSVVIVSPQDIDGRKGSMNELEVENFVKALNSLKVKPEVIYIDSADVKAERFAENIRSRLAYEAKVVAEHKADAKYEIVSAASILAKVIRDREIEKLKAEYGDFGSGYPSDPRTKKWLEEWYSKHGNFPPIVRRTWDTAKKIEEKFKRAQLTLDNFLKRFRN

SEQ ID NO: 199 - protein, 224 aa, Artificial Sequence
  Synthetic
MKVAGADEAGRGTVIGPLVIVAAVVEEDKIRSLTKLGVKDSKQLTPAQREKLFDEIVKVLDDYSVVIVSPQDIDGRKGSMNELEVENFVKALNSLKVKPEVIYIDSADVKAERFAENIRSRLAYEAKVVAEHKADAKYEIVSAASILAKVIRDREIEKLKAEYGDFGSGYPSDPRTKKWLEEWYSKHGNFPPIVRRTWDTAKKIEEKFKRAQLTLDNFLKRFRN

SEQ ID NO: 200 - DNA, 22 bp, Artificial Sequence
  Synthetic
cagcctcatccaaaagaggaaa

SEQ ID NO: 201 - DNA, 21 bp, Artificial Sequence
  Synthetic
ctcactctaaaccccagcatt

SEQ ID NO: 202 - DNA, 27 bp, Artificial Sequence
  Synthetic
  misc_feature (23)..(23): RNA base
  misc_feature (27)..(27): 3' C3 spacer (propanediol) blocker group
cagcctcatccaaaagaggaaacagga

SEQ ID NO: 203 - DNA, 27 bp, Artificial Sequence
  Synthetic
  misc_feature (23)..(23): RNA base
  misc_feature (27)..(27): 3' C3 spacer (propanediol) blocker group
cagcctcatccaaaagaggaaauagga

SEQ ID NO: 204 - DNA, 22 bp, Artificial Sequence
  Synthetic
gtgattttggtctagctacagt

SEQ ID NO: 205 - DNA, 23 bp, Artificial Sequence
  Synthetic
cctcaattcttaccatccacaaa

SEQ ID NO: 206 - DNA, 28 bp, Artificial Sequence
  Synthetic
  misc_feature (23)..(23): RNA base
  misc_feature (28)..(28): 3' C3 spacer (propanediol) blocker group
gtgattttggtctagctacagtgaaatg

SEQ ID NO: 207 - DNA, 28 bp, Artificial Sequence
  Synthetic
  misc_feature (23)..(23): RNA base
  misc_feature (28)..(28): 3' C3 spacer (propanediol) blocker group
gtgattttggtctagctacagagaaatg

SEQ ID NO: 208 - DNA, 401 bp, Artificial Sequence
  Synthetic
taagaggaaagatgaagtactatgttttaaagaatattatattacagaattatagaaattagatctcttacctaaactcttcataatgcttgctctgataggaaaatgagatctactgttttcctttacttactacacctcagatatatttcttcatgaagacctcacagtaaaaataggtgattttggtctagctacagtgaaatctcgatggagtgggtcccatcagtttgaacagttgtctggatccattttgtggatggtaagaattgaggctatttttccactgattaaatttttggccctgagatgctgctgagttactagaaagtcattgaaggtctcaactatagtattttcatagttcccagtattcacaaaaatcagtgttcttatttttt

SEQ ID NO: 209 - DNA, 401 bp, Artificial Sequence
  Synthetic
taagaggaaagatgaagtactatgttttaaagaatattatattacagaattatagaaattagatctcttacctaaactcttcataatgcttgctctgataggaaaatgagatctactgttttcctttacttactacacctcagatatatttcttcatgaagacctcacagtaaaaataggtgattttggtctagctacagagaaatctcgatggagtgggtcccatcagtttgaacagttgtctggatccattttgtggatggtaagaattgaggctatttttccactgattaaatttttggccctgagatgctgctgagttactagaaagtcattgaaggtctcaactatagtattttcatagttcccagtattcacaaaaatcagtgttcttatttttt

SEQ ID NO: 210 - DNA, 26 bp, Artificial Sequence
  Synthetic
  misc_feature (21)..(21): RNA base
  misc_feature (26)..(26): 3' C3 spacer (propanediol) blocker group
gtgattttggtctagctacagtaaaa

SEQ ID NO: 211 - DNA, 26 bp, Artificial Sequence
  Synthetic
  misc_feature (21)..(21): RNA base
  misc_feature (26)..(26): 3' C3 spacer (propanediol) blocker group
gtgattttggtctagctacagaaaaa

SEQ ID NO: 212 - DNA, 53 bp, Artificial Sequence
  Synthetic
agccgaatacggtgattttggttccgcatacccgtctgatccgcgtactaaga

SEQ ID NO: 213 - DNA, 53 bp, Artificial Sequence
  Synthetic
tcttagtacgcggatcagacgggtatgcggaaccaaaatcaccgtattcggct

SEQ ID NO: 214 - protein, 224 aa, Artificial Sequence
  Synthetic
MKVAGADEAGRGPVIGPLVIVAAVVEEDKIRSLTKLGVKDSKQLTPAQREKLFDEIVKVLDDYSVVIVSPQDIDGRKGSMNELEVENFVKALNSLKVKPEVIYIDSADVKAERFAENIRSRLAYEAKVVAEHKADAKYEIVSAASILAKVIRDREIEKLKAEYGDFGSAYPSDPRTKKWLEEWYSKHGNFPPIVRRTWDTAKKIEEKFKRAQLTLDNFLKRFRN

SEQ ID NO: 215 - DNA, 22 bp, Artificial Sequence
  Synthetic
cagcctcatccaaaagaggaaa

SEQ ID NO: 216 - DNA, 21 bp, Artificial Sequence
  Synthetic
ctcactctaaaccccagcatt

SEQ ID NO: 217 - DNA, 27 bp, Artificial Sequence
  Synthetic
  misc_feature (23)..(23): RNA base
  misc_feature (27)..(27): 3' C3 spacer (propanediol) blocker group
cagcctcatccaaaagaggaaacagga

SEQ ID NO: 218 - DNA, 27 bp, Artificial Sequence
  Synthetic
  misc_feature (23)..(23): RNA base
  misc_feature (27)..(27): 3' C3 spacer (propanediol) blocker group
cagcctcatccaaaagaggaaauagga